European Patent Application EP 4 410 307 A1, published August 7, 2024. Title: PYRROLO BENZODIAZEPINE DERIVATIVE, AND CONJUGATE, PREPARATION METHOD AND USE THEREOF. Applicant: JIANGSU HENGRUI PHARMACEUTICALS CO., LTD. Application CN. The sequence listing filed with the application follows.

SEQUENCE LISTING (7 sequences)

SEQ ID NO: 1 - protein, 214 aa, synthetic construct
DIQMTQSPSSLSASVGDRVTITCRASQDVNTAVAWYQQKPGKAPKLLIYSASFLYSGVPSRFSGSRSGTDFTLTISSLQPEDFATYYCQQHYTTPPTFGQGTKVEIKRTVAAPSVFIFPPSDEQLKSGTASVVCLLNNFYPREAKVQWKVDNALQSGNSQESVTEQDSKDSTYSLSSTLTLSKADYEKHKVYACEVTHQGLSSPVTKSFNRGEC

SEQ ID NO: 2 - protein, 450 aa, synthetic construct
EVQLVESGGGLVQPGGSLRLSCAASGFNIKDTYIHWVRQAPGKGLEWVARIYPTNGYTRYADSVKGRFTISADTSKNTAYLQMNSLRAEDTAVYYCSRWGGDGFYAMDYWGQGTLVTVSSASTKGPSVFPLAPSSKSTSGGTAALGCLVKDYFPEPVTVSWNSGALTSGVHTFPAVLQSSGLYSLSSVVTVPSSSLGTQTYICNVNHKPSNTKVDKKVEPKSCDKTHTCPPCPAPELLGGPSVFLFPPKPKDTLMISRTPEVTCVVVDVSHEDPEVKFNWYVDGVEVHNAKTKPREEQYNSTYRVVSVLTVLHQDWLNGKEYKCKVSNKALPAPIEKTISKAKGQPREPQVYTLPPSREEMTKNQVSLTCLVKGFYPSDIAVEWESNGQPENNYKTTPPVLDSDGSFFLYSKLTVDKSRWQQGNVFSCSVMHEALHNHYTQKSLSLSPGK

SEQ ID NO: 3 - protein, 220 aa, synthetic construct
DIVLTQSPDSLAVSLGERATINCKSSQSLLNSGNQKNYLTWYQQKPGQPPKLLIYWASTRESGVPDRFSGSGSGTDFTLTISSLQAEDVAVYYCQNAYTYPFTFGQGTKLEIKRTVAAPSVFIFPPSDEQLKSGTASVVCLLNNFYPREAKVQWKVDNALQSGNSQESVTEQDSKDSTYSLSSTLTLSKADYEKHKVYACEVTHQGLSSPVTKSFNRGEC

SEQ ID NO: 4 - protein, 448 aa, synthetic construct
EVQLVQSGAEVKKPGASVKVSCKASGYTFTSYWMHWVRQAPGQRLEWMGMIHPNSGSTNYNEKFKGRVTITRDTSASTAYMELSSLRSEDTAVYYCARLKTGNSFDYWGQGTTVTVSSASTKGPSVFPLAPSSKSTSGGTAALGCLVKDYFPEPVTVSWNSGALTSGVHTFPAVLQSSGLYSLSSVVTVPSSSLGTQTYICNVNHKPSNTKVDKKVEPKSCDKTHTCPPCPAPELLGGPSVFLFPPKPKDTLMISRTPEVTCVVVDVSHEDPEVKFNWYVDGVEVHNAKTKPREEQYNSTYRVVSVLTVLHQDWLNGKEYKCKVSNKALPAPIEKTISKAKGQPREPQVYTLPPSRDELTKNQVSLTCLVKGFYPSDIAVEWESNGQPENNYKTTPPVLDSDGSFFLYSKLTVDKSRWQQGNVFSCSVMHEALHNHYTQKSLSLSPGK

SEQ ID NO: 5 - protein, 215 aa, synthetic construct
DIQMTQSPSSLSASIGDRATITCRASQHVGTYLNWYQQKPGKTPKLLISGAANLQSGVPSRFSGSGSGTDFTLTISSLQPEDFATYYCQQSYNTPPFSFGQGTKVEIKRTVAAPSVFIFPPSDEQLKSGTASVVCLLNNFYPREAKVQWKVDNALQSGNSQESVTEQDSKDSTYSLSSTLTLSKADYEKHKVYACEVTHQGLSSPVTKSFNRGEC

SEQ ID NO: 6 - protein, 447 aa, synthetic construct
QVQLVQSGGGLVQPGRSLRLSCAASGFTFDDYAMHWVRQAPGKGLEWVSGISWNSGSIGYADSVKGRFTISRDNAKNSLYLQMNSLRAEDTALYYCAKEGLPGLDYWGQGTLVTVSSASTKGPSVFPLAPSSKSTSGGTAALGCLVKDYFPEPVTVSWNSGALTSGVHTFPAVLQSSGLYSLSSVVTVPSSSLGTQTYICNVNHKPSNTKVDKKVEPKSCDKTHTCPPCPAPELLGGPSVFLFPPKPKDTLMISRTPEVTCVVVDVSHEDPEVKFNWYVDGVEVHNAKTKPREEQYNSTYRVVSVLTVLHQDWLNGKEYKCKVSNKALPAPIEKTISKAKGQPREPQVYTLPPSRDELTKNQVSLTCLVKGFYPSDIAVEWESNGQPENNYKTTPPVLDSDGSFFLYSKLTVDKSRWQQGNVFSCSVMHEALHNHYTQKSLSLSPGK

SEQ ID NO: 7 - protein, 261 aa, synthetic construct
MAVTACQGLGFVVSLIGIAGIIAATCMDQWSTQDLYNNPVTAVFNYQGLWRSCVRESSGFTECRGYFTLLGLPAMLQAVRALMIVGIVLGAIGLLVSIFALKCIRIGSMEDSAKANMTLTSGIMFIVSGLCAIAGVSVFANMLVTNFWMSTANMYTGMGGMVQTVQTRYTFGAALFVGWVAGGLTLIGGVMMCIACRGLAPEETNYKAVSYHASGHSVAYKPGGFKASTGFGSNTKNKKIYDGGARTEDEVQSYPSKHDYV